European Patent Specification EP 4 045 083 B1, published January 10, 2024. Title: COMBINATION THERAPIES FOR TREATING MYELODYSPLASTIC SYNDROMES AND ACUTE MYELOID LEUKEMIA. Applicant: FORTY SEVEN, INC. The sequence listing filed with the application follows.

SEQUENCE LISTING (153 sequences)

SEQ ID NO: 1 - protein, 5 aa, Artificial Sequence
  source: /note="Description of Artificial Sequence: Synthetic peptide"
SYWIT

SEQ ID NO: 2 - protein, 17 aa, Artificial Sequence
  source: /note="Description of Artificial Sequence: Synthetic peptide"
DIYPGSGSTNHIEKFKS

SEQ ID NO: 3 - protein, 11 aa, Artificial Sequence
  source: /note="Description of Artificial Sequence: Synthetic peptide"
GYGSSYGYFDY

SEQ ID NO: 4 - protein, 11 aa, Artificial Sequence
  source: /note="Description of Artificial Sequence: Synthetic peptide"
RASENIYSYLA

SEQ ID NO: 5 - protein, 7 aa, Artificial Sequence
  source: /note="Description of Artificial Sequence: Synthetic peptide"
TAKTLAE

SEQ ID NO: 6 - protein, 9 aa, Artificial Sequence
  source: /note="Description of Artificial Sequence: Synthetic peptide"
QHQYGPPFT

SEQ ID NO: 7 - protein, 120 aa, Artificial Sequence
  source: /note="Description of Artificial Sequence: Synthetic polypeptide"
QVQLVQSGAEVKKPGASVKVSCKASGYTFTSYWITWVKQAPGQGLEWIGDIYPGSGSTNHIEKFKSKATLTVDTSISTAYMELSRLRSDDTAVYYCATGYGSSYGYFDYWGQGTLVTVSS

SEQ ID NO: 8 - protein, 107 aa, Artificial Sequence
  source: /note="Description of Artificial Sequence: Synthetic polypeptide"
DIQMTQSPSSLSASVGDRVTITCRASENIYSYLAWYQQKPGKAPKLLIYTAKTLAEGVPSRFSGSGSGTDFTLTISSLQPEDFATYYCQHQYGPPFTFGQGTKLEIK

SEQ ID NO: 9 - protein, 5 aa, Artificial Sequence
  source: /note="Description of Artificial Sequence: Synthetic peptide"
SYWMH

SEQ ID NO: 10 - protein, 17 aa, Artificial Sequence
  source: /note="Description of Artificial Sequence: Synthetic peptide"
NIDPSDSDTHYNQKFKD

SEQ ID NO: 11 - protein, 10 aa, Artificial Sequence
  source: /note="Description of Artificial Sequence: Synthetic peptide"
GYSKYYAMDY

SEQ ID NO: 12 - protein, 16 aa, Artificial Sequence
  source: /note="Description of Artificial Sequence: Synthetic peptide"
RSSQSIVHSYGNTYLE

SEQ ID NO: 13 - protein, 7 aa, Artificial Sequence
  source: /note="Description of Artificial Sequence: Synthetic peptide"
KVSNRFS

SEQ ID NO: 14 - protein, 9 aa, Artificial Sequence
  source: /note="Description of Artificial Sequence: Synthetic peptide"
FQGSHVPYT

SEQ ID NO: 15 - protein, 119 aa, Artificial Sequence
  source: /note="Description of Artificial Sequence: Synthetic polypeptide"
QVQLVQSGAEVKKPGASVKVSCKASGYTFTSYWMHWVRQAPGQGLEWMGNIDPSDSDTHYNQKFKDRVTMTRDTSTSTVYMELSSLRSEDTAVYYCARGYSKYYAMDYWGQGTLVTVSS

SEQ ID NO: 16 - protein, 112 aa, Artificial Sequence
  source: /note="Description of Artificial Sequence: Synthetic polypeptide"
DIVMTQTPLSLSVTPGQPASISCRSSQSIVHSYGNTYLEWYLQKPGQSPQLLIYKVSNRFSGVPDRFSGSGSGTDFTLKISRVEAEDVGVYYCFQGSHVPYTFGQGTKLEIK

SEQ ID NO: 17 - protein, 449 aa, Artificial Sequence
  source: /note="Description of Artificial Sequence: Synthetic polypeptide"
QVQLVQSGAEVKKPGASVKVSCKASGYTFTSYWITWVKQAPGQGLEWIGDIYPGSGSTNHIEKFKSKATLTVDTSISTAYMELSRLRSDDTAVYYCATGYGSSYGYFDYWGQGTLVTVSSASTKGPSVFPLAPSSKSTSGGTAALGCLVKDYFPEPVTVSWNSGALTSGVHTFPAVLQSSGLYSLSSVVTVPSSSLGTQTYICNVNHKPSNTKVDKKVEPKSCDKTHTCPPCPAPELLGGPSVFLFPPKPKDTLMISRTPEVTCVVVDVSHEDPEVKFNWYVDGVEVHNAKTKPREEQYASTYRVVSVLTVLHQDWLNGKEYKCKVSNKALPAPIEKTISKAKGQPREPQVYTLPPSREEMTKNQVSLTCLVKGFYPSDIAVEWESNGQPENNYKTTPPVLDSDGSFFLYSKLTVDKSRWQQGNVFSCSVMHEALHNHYTQKSLSLSPG

SEQ ID NO: 18 - protein, 214 aa, Artificial Sequence
  source: /note="Description of Artificial Sequence: Synthetic polypeptide"
DIQMTQSPSSLSASVGDRVTITCRASENIYSYLAWYQQKPGKAPKLLIYTAKTLAEGVPSRFSGSGSGTDFTLTISSLQPEDFATYYCQHQYGPPFTFGQGTKLEIKRTVAAPSVFIFPPSDEQLKSGTASVVCLLNNFYPREAKVQWKVDNALQSGNSQESVTEQDSKDSTYSLSSTLTLSKADYEKHKVYACEVTHQGLSSPVTKSFNRGEC

SEQ ID NO: 19 - protein, 448 aa, Artificial Sequence
  source: /note="Description of Artificial Sequence: Synthetic polypeptide"
QVQLVQSGAEVKKPGASVKVSCKASGYTFTSYWMHWVRQAPGQGLEWMGNIDPSDSDTHYNQKFKDRVTMTRDTSTSTVYMELSSLRSEDTAVYYCARGYSKYYAMDYWGQGTLVTVSSASTKGPSVFPLAPSSKSTSGGTAALGCLVKDYFPEPVTVSWNSGALTSGVHTFPAVLQSSGLYSLSSVVTVPSSSLGTQTYICNVNHKPSNTKVDKKVEPKSCDKTHTCPPCPAPELLGGPSVFLFPPKPKDTLMISRTPEVTCVVVDVSHEDPEVKFNWYVDGVEVHNAKTKPREEQYASTYRVVSVLTVLHQDWLNGKEYKCKVSNKALPAPIEKTISKAKGQPREPQVYTLPPSREEMTKNQVSLTCLVKGFYPSDIAVEWESNGQPENNYKTTPPVLDSDGSFFLYSKLTVDKSRWQQGNVFSCSVMHEALHNHYTQKSLSLSPG

SEQ ID NO: 20 - protein, 219 aa, Artificial Sequence
  source: /note="Description of Artificial Sequence: Synthetic polypeptide"
DIVMTQTPLSLSVTPGQPASISCRSSQSIVHSYGNTYLEWYLQKPGQSPQLLIYKVSNRFSGVPDRFSGSGSGTDFTLKISRVEAEDVGVYYCFQGSHVPYTFGQGTKLEIKRTVAAPSVFIFPPSDEQLKSGTASVVCLLNNFYPREAKVQWKVDNALQSGNSQESVTEQDSKDSTYSLSSTLTLSKADYEKHKVYACEVTHQGLSSPVTKSFNRGEC

SEQ ID NO: 21 - protein, 5 aa, Artificial Sequence
  source: /note="Description of Artificial Sequence: Synthetic peptide"
DYYIH

SEQ ID NO: 22 - protein, 17 aa, Artificial Sequence
  source: /note="Description of Artificial Sequence: Synthetic peptide"
RIDPEDGETKYAPKFQG

SEQ ID NO: 23 - protein, 5 aa, Artificial Sequence
  source: /note="Description of Artificial Sequence: Synthetic peptide"
GGFAY

SEQ ID NO: 24 - protein, 11 aa, Artificial Sequence
  source: /note="Description of Artificial Sequence: Synthetic peptide"
ASSSVSSSYLY

SEQ ID NO: 25 - protein, 7 aa, Artificial Sequence
  source: /note="Description of Artificial Sequence: Synthetic peptide"
STSNLAS

SEQ ID NO: 26 - protein, 9 aa, Artificial Sequence
  source: /note="Description of Artificial Sequence: Synthetic peptide"
HQWSSHPYT

SEQ ID NO: 27 - protein, 114 aa, Artificial Sequence
  source: /note="Description of Artificial Sequence: Synthetic polypeptide"
EVQLQQSGAELVKPGASVKLSCTASGFNIKDYYIHWVKQRTEQGLEWIGRIDPEDGETKYAPKFQGKATITADTSSNTAYLQLNSLTSEDTAVYSCAKGGFAYWGQGTLVTVSA

SEQ ID NO: 28 - protein, 108 aa, Artificial Sequence
  source: /note="Description of Artificial Sequence: Synthetic polypeptide"
QIVLTQSPAIMSASPGEKVTLTCSASSSVSSSYLYWYQQKPGSSPKLWIYSTSNLASGVPARFSGSGSGTSYSLTISSMEAEDAASYFCHQWSSHPYTFGGGTKLEIK

SEQ ID NO: 29 - protein, 5 aa, Artificial Sequence
  source: /note="Description of Artificial Sequence: Synthetic peptide"
SYWMH

SEQ ID NO: 30 - protein, 17 aa, Artificial Sequence
  source: /note="Description of Artificial Sequence: Synthetic peptide"
NIDPSDSDTHYNQKFKD

SEQ ID NO: 31 - protein, 12 aa, Artificial Sequence
  source: /note="Description of Artificial Sequence: Synthetic peptide"
SYGNYGENAMDY

SEQ ID NO: 32 - protein, 16 aa, Artificial Sequence
  source: /note="Description of Artificial Sequence: Synthetic peptide"
RSSQSIVHSYGNTYLE

SEQ ID NO: 33 - protein, 7 aa, Artificial Sequence
  source: /note="Description of Artificial Sequence: Synthetic peptide"
KVSNRFS

SEQ ID NO: 34 - protein, 9 aa, Artificial Sequence
  source: /note="Description of Artificial Sequence: Synthetic peptide"
FQGSHVPFT

SEQ ID NO: 35 - protein, 120 aa, Artificial Sequence
  source: /note="Description of Artificial Sequence: Synthetic polypeptide"
QVKLQESGAELVRPGSSVKLSCKASGYTFTSYWMHWVKQRPIQGLEWIGNIDPSDSDTHYNQKFKDKATLTVDNSSSTAYMQLSSLTSEDSAVYYCASYGNYGENAMDYWGQGTSVTVSS

SEQ ID NO: 36 - protein, 112 aa, Artificial Sequence
  source: /note="Description of Artificial Sequence: Synthetic polypeptide"
DILMTQTPLSLPVSLGDQASISCRSSQSIVHSYGNTYLEWYLQKPGQSPKLLIYKVSNRFSGVPDRFSGSGSGTDFTLKISRVEAEDLGVYYCFQGSHVPFTFGSGTKLEIK

SEQ ID NO: 37 - DNA, 1347 bp, Artificial Sequence
  source: /note="Description of Artificial Sequence: Synthetic polynucleotide"
caggttcagttggttcagtctggcgccgaagtgaagaaacctggcgcctctgtgaaggtgtcctgcaaggcttccggctacacctttaccagctactggatcacctgggtcaagcaggctcctggacagggactcgagtggatcggcgatatctatcctggctccggctccaccaaccacatcgagaagttcaagtccaaggctaccctgaccgtggacacctccatctccaccgcctacatggaactgtcccggctgagatctgacgacaccgccgtgtactattgcgctaccggctacggctcctcctacggctactttgattattggggccagggcaccctggtcaccgtgtcctctgcttctaccaagggacccagcgtgttccctctggctccttccagcaagtctacctctggcggaacagctgctctgggctgcctggtcaaggactactttcctgagcctgtgaccgtgtcttggaactctggcgctctgacatctggcgtgcacacattccctgctgtgctgcagtcctccggcctgtactctctgtcctctgtcgtgaccgtgccttccagctctctgggaacccagacctacatctgcaatgtgaaccacaagccttccaacaccaaggtggacaagaaggtggaacccaagtcctgcgacaagacccacacctgtcctccatgtcctgctccagaactgctcggcggaccttccgtgtttctgttccctccaaagcctaaggacaccctgatgatctctcggacccctgaagtgacctgcgtggtggtggatgtgtctcacgaggacccagaagtgaagttcaattggtacgtggacggcgtggaagtgcacaacgccaagaccaagcctagagaggaacagtacgcctccacctacagagtggtgtccgtgctgacagtgctgcaccaggattggctgaacggcaaagagtacaagtgcaaggtgtccaacaaggccctgcctgctcctatcgaaaagaccatctccaaggccaagggccagcctagggaaccccaggtttacaccctgccacctagccgggaagagatgaccaagaaccaggtgtccctgacctgcctcgtgaagggcttctacccttccgatatcgctgtggaatgggagagcaacggccagcctgagaacaactacaagacaacccctcctgtgctggactccgacggctcattctttctgtactccaagctgactgtggacaagtccagatggcagcagggcaacgtgttctcctgcagcgtgatgcacgaggccctgcacaatcactacacacagaagtctctgtctctgagccccggc

SEQ ID NO: 38 - DNA, 642 bp, Artificial Sequence
  source: /note="Description of Artificial Sequence: Synthetic polynucleotide"
gacatccagatgacccagtctccatcctctctgtccgcctctgtgggcgacagagtgaccatcacctgtcgggcctccgagaacatctactcctacctggcctggtatcagcagaagcctggcaaggctcccaagctgctgatctacaccgctaagacactggccgagggcgtgccctctagattttctggctctggaagcggcaccgactttaccctgacaatctccagcctgcagcctgaggacttcgccacctactactgccagcaccagtacggccctccattcacctttggccagggcaccaagctggaaatcaagcggacagtggccgctccttccgtgttcatcttcccaccttccgacgagcagctgaagtctggcacagcctctgtcgtgtgcctgctgaacaacttctaccctcgggaagccaaggtgcagtggaaggtggacaatgccctgcagtccggcaactcccaagagtctgtgaccgagcaggactccaaggacagcacctacagcctgtcctccacactgaccctgtccaaggccgactacgagaagcacaaggtgtacgcctgcgaagtgacccatcagggcctgtctagccctgtgaccaagtctttcaaccggggcgagtgc

SEQ ID NO: 39 - DNA, 1344 bp, Artificial Sequence
  source: /note="Description of Artificial Sequence: Synthetic polynucleotide"
caggttcagttggttcagtctggcgccgaagtgaagaaacctggcgcctctgtgaaggtgtcctgcaaggcttccggctacacctttaccagctactggatgcactgggtccgacaggctccaggacaaggcttggagtggatgggcaacatcgacccctctgacagcgacacccactacaaccagaaattcaaggaccgcgtgaccatgaccagagacacctccaccagcaccgtgtacatggaactgtccagcctgagatccgaggacaccgccgtgtactactgtgccagaggctactccaagtactacgccatggactactggggccagggcacactggttaccgtgtcctctgcttccaccaagggaccctctgtgttccctctggctccttccagcaagtctacctctggcggaacagctgctctgggctgcctggtcaaggactactttcctgagcctgtgaccgtgtcttggaactctggcgctctgacatctggcgtgcacacattccctgctgtgctgcagtcctccggcctgtactctctgtcctctgtcgtgaccgtgccttccagctctctgggaacccagacctacatctgcaatgtgaaccacaagccttccaacaccaaggtggacaagaaggtggaacccaagtcctgcgacaagacccacacctgtcctccatgtcctgctccagaactgctcggcggaccttccgtgtttctgttccctccaaagcctaaggacaccctgatgatctctcggacccctgaagtgacctgcgtggtggtggatgtgtcccacgaagatccagaagtgaagttcaattggtacgtggacggcgtggaagtgcacaacgccaagaccaagcctagagaggaacagtacgcctccacctacagagtggtgtccgtgctgacagtgctgcaccaggattggctgaacggcaaagagtacaagtgcaaggtgtccaacaaggccctgcctgctcctatcgaaaagaccatctccaaggccaagggccagcctagggaaccccaggtttacaccctgcctccaagccgggaagagatgaccaagaaccaggtgtccctgacctgcctcgtgaagggcttctacccttccgatatcgccgtggaatgggagagcaatggccagccagagaacaactacaagacaacccctcctgtgctggactccgacggctcattctttctgtactccaagctgaccgtggacaagtccagatggcagcagggcaacgtgttctcctgcagcgtgatgcacgaggccctgcacaatcactatacccagaagtccctgtctctgtcccctggc

SEQ ID NO: 40 - DNA, 657 bp, Artificial Sequence
  source: /note="Description of Artificial Sequence: Synthetic polynucleotide"
gacatcgtgatgacccagacacctctgagcctgagcgtgacacctggacagcctgcctccatctcctgcagatcctctcagtccatcgtgcactcctacggcaacacctacctggaatggtatctgcagaagcccggccagtctcctcagctgctgatctacaaggtgtccaaccggttctctggcgtgcccgacagattttccggctctggctctggcaccgacttcaccctgaagatctccagagtggaagccgaggacgtgggcgtgtactactgcttccaaggctctcacgtgccctacacctttggccagggcaccaagctggaaatcaagcggacagtggccgctccttccgtgttcatcttcccaccttccgacgagcagctgaagtccggcacagcttctgtcgtgtgcctgctgaacaacttctaccctcgggaagccaaggtgcagtggaaggtggacaatgccctgcagtccggcaactcccaagagtctgtgaccgagcaggactccaaggacagcacctacagcctgtccagcacactgaccctgtccaaggccgactacgagaagcacaaggtgtacgcctgcgaagtgacccatcagggcctgtctagccctgtgaccaagtctttcaaccggggcgagtgc

SEQ ID NO: 41 - DNA, 342 bp, Artificial Sequence
  source: /note="Description of Artificial Sequence: Synthetic polynucleotide"
gaggttcagctgcagcagtctggggcagagcttgtgaagccaggggcctcagtcaagttgtcctgcacagcttctggcttcaacattaaagactactatatacactgggtgaagcagaggactgaacagggcctggagtggattggaaggattgatcctgaggatggtgaaactaaatatgccccgaaattccagggcaaggccactataacagcagacacatcctccaacacagcctacctgcagctcaacagcctgacatctgaggacactgccgtctattcctgtgctaagggggggtttgcttactggggccaagggactctggtcactgtctctgca

SEQ ID NO: 42 - DNA, 324 bp, Artificial Sequence
  source: /note="Description of Artificial Sequence: Synthetic polynucleotide"
caaattgttctcacccagtctccagcaatcatgtctgcatctcctggggagaaggtcaccttgacctgcagtgccagttcaagtgtaagttccagctacttgtactggtaccagcagaagccaggatcctcccccaaactctggatttatagcacatccaacctggcttctggagtccctgctcgcttcagtggcagtgggtctgggacctcttactctctcacaatcagcagcatggaggctgaagatgctgcctcttatttctgccatcagtggagtagtcacccgtacacgttcggaggggggaccaagctggaaataaaa

SEQ ID NO: 43 - DNA, 360 bp, Artificial Sequence
  source: /note="Description of Artificial Sequence: Synthetic polynucleotide"
caggtcaagctgcaggagtctggggctgagctggtgaggcctgggtcttcagtgaagctgtcctgcaaggcttctggctacaccttcaccagctactggatgcattgggtgaagcagaggcctatacaaggccttgaatggattggtaacattgacccttctgatagtgatactcactacaatcaaaagttcaaggacaaggccacattgactgtggacaactcctccagcacagcctacatgcagctcagcagcctgacctctgaggactctgcggtctattactgtgcaagctatggtaactacggggagaatgctatggactactggggtcaaggaacctcagtcaccgtctcctca

SEQ ID NO: 44 - DNA, 336 bp, Artificial Sequence
  source: /note="Description of Artificial Sequence: Synthetic polynucleotide"
gatattttgatgacccaaactccactctccctgcctgtcagtcttggagatcaagcctccatctcttgcagatctagtcagagcattgtacatagttatggaaacacctatttagaatggtacctgcagaaaccaggccagtctccaaaactcctgatctacaaagtttccaaccgattttctggggtcccagacaggttcagtggcagtggatcaggtacagatttcacactcaagatcagcagagtggaggctgaggatctgggagtttattactgctttcaaggttcacatgttccattcacgttcggctcggggacaaagttggaaataaaa

SEQ ID NO: 45 - protein, 116 aa, Homo sapiens
EEELQVIQPDKSVLVAAGETATLRCTATSLIPVGPIQWFRGAGPGRELIYNQKEGHFPRVTTVSDLTKRNNMDFSIRIGNITPADAGTYYCVKFRKGSPDDVEFKSGAGTELSVRA

SEQ ID NO: 46 - protein, 113 aa, Artificial Sequence
  source: /note="Description of Artificial Sequence: Synthetic polypeptide"
EVQLVQSGAEVKKPGATVKISCKVSGFNIKDYYIHWVQQAPGKGLEWIGRIDPEDGETKYAPKFQDRATITADTSTDTAYMELSSLRSEDTAVYYCARWGAYWGQGTLVTVSS

SEQ ID NO: 47 - protein, 108 aa, Artificial Sequence
  source: /note="Description of Artificial Sequence: Synthetic polypeptide"
QIVLTQSPPTLSLSPGERVTLTCSASSSVSSSYLYWYQQKPGQAPKLWIYSTSNLASGVPARFSGSGSGTSYTLTISSLQPEDFAVYFCHQWSSYPRTFGAGTKLEIK

SEQ ID NO: 48 - protein, 116 aa, Homo sapiens; identical to SEQ ID NO: 45

SEQ ID NO: 49 - protein, 115 aa, Homo sapiens
EEELQVIQPDKSVSVAAGESAILHCTVTSLIPVGPIQWFRGAGPARELIYNQKEGHFPRVTTVSESTKRENMDFSISISNITPADAGTYYCVKFRKGSPDTEFKSGAGTELSVRA

SEQ ID NO: 50 - protein, 444 aa, Artificial Sequence
  source: /note="Description of Artificial Sequence: Synthetic polypeptide"
QVQLVQSGAEVKKPGASVKVSCKASGYTFTNYNMHWVRQAPGQRLEWMGTIYPGNDDTSYNQKFKDRVTITADTSASTAYMELSSLRSEDTAVYYCARGGYRAMDYWGQGTLVTVSSASTKGPSVFPLAPCSRSTSESTAALGCLVKDYFPEPVTVSWNSGALTSGVHTFPAVLQSSGLYSLSSVVTVPSSSLGTKTYTCNVDHKPSNTKVDKRVESKYGPPCPPCPAPEFLGGPSVFLFPPKPKDTLMISRTPEVTCVVVDVSQEDPEVQFNWYVDGVEVHNAKTKPREEQFNSTYRVVSVLTVLHQDWLNGKEYKCKVSNKGLPSSIEKTISKAKGQPREPQVYTLPPSQEEMTKNQVSLTCLVKGFYPSDIAVEWESNGQPENNYKTTPPVLDSDGSFFLYSRLTVDKSRWQEGNVFSCSVMHEALHNHYTQKSLSLSLGK

SEQ ID NO: 51 - protein, 219 aa, Artificial Sequence
  source: /note="Description of Artificial Sequence: Synthetic polypeptide"
DIVMTQSPLSLPVTPGEPASISCRSSQSIVYSNGNTYLGWYLQKPGQSPQLLIYKVSNRFSGVPDRFSGSGSGTDFTLKISRVEAEDVGVYYCFQGSHVPYTFGQGTKLEIKRTVAAPSVFIFPPSDEQLKSGTASVVCLLNNFYPREAKVQWKVDNALQSGNSQESVTEQDSKDSTYSLSSTLTLSKADYEKHKVYACEVTHQGLSSPVTKSFNRGEC

SEQ ID NO: 52 - protein, 5 aa, Artificial Sequence
  source: /note="Description of Artificial Sequence: Synthetic peptide"
NYNMH

SEQ ID NO: 53 - protein, 17 aa, Artificial Sequence
  source: /note="Description of Artificial Sequence: Synthetic peptide"
TIYPGNDDTSYNQKFKD

SEQ ID NO: 54 - protein, 8 aa, Artificial Sequence
  source: /note="Description of Artificial Sequence: Synthetic peptide"
GGYRAMDY

SEQ ID NO: 55 - protein, 15 aa, Artificial Sequence
  source: /note="Description of Artificial Sequence: Synthetic peptide"
RSSQSIVYSNGNTYL

SEQ ID NO: 56 - protein, 7 aa, Artificial Sequence
  source: /note="Description of Artificial Sequence: Synthetic peptide"
KVSNRFS

SEQ ID NO: 57 - protein, 9 aa, Artificial Sequence
  source: /note="Description of Artificial Sequence: Synthetic peptide"
FQGSHVPYT

SEQ ID NO: 58 - protein, 116 aa, Artificial Sequence
  source: /note="Description of Artificial Sequence: Synthetic polypeptide"
QVQLQQPGAELVKPGASVMMSCKASGYTFTNYNMHWVKQTPGQGLEWIGTIYPGNDDTSYNQKFKDKATLTADKSSSAAYMQLSSLTSEDSAVYYCARGGYRAMDYWGQTSVTVSS

SEQ ID NO: 59 - protein, 112 aa, Artificial Sequence
  source: /note="Description of Artificial Sequence: Synthetic polypeptide"
DVLMTQTPLSLPVSLGDQASISCRSSQSIVYSNGNTYLGWYLQKPGQSPKLLIYKVSNRFSGVPDRFSGSGSGTDFTLKISRVEAEDLGVYHCFQGSHVPYTFGGGTKVEIK

SEQ ID NO: 60 - protein, 118 aa, Artificial Sequence
  source: /note="Description of Artificial Sequence: Synthetic polypeptide"
EVQLVESGGGLVQPGGSLRLSCAASGFTFSGYGMSWVRQAPGKGLEWVATITSGGTYTYYPDSVKGRFTISRDNAKNSLYLQMNSLRAEDTAVYYCARSLAGNAMDYWGQGTLVTVSS

SEQ ID NO: 61 - protein, 107 aa, Artificial Sequence
  source: /note="Description of Artificial Sequence: Synthetic polypeptide"
EIVLTQSPATLSLSPGERATLSCRASQTISDYLHWYQQKPGQAPRLLIKFASQSISGIPARFSGSGSGTDFTLTISSLEPEDFAVYYCQNGHGFPRTFGQGTKVEIK

SEQ ID NO: 62 - protein, 109 aa, Artificial Sequence
  source: /note="Description of Artificial Sequence: Synthetic polypeptide"
EVQLVESGGGLVQPGGSLRLSCAASGFTFSSYWMSWVRQAPGKGLEWVANIKQDGSEKYYVDSVKGRFTISRDNAKNSLYLQMNSLRAEDTAVYYCARWGQGTLVTVSS

SEQ ID NO: 63 - protein, 107 aa, Artificial Sequence
  source: /note="Description of Artificial Sequence: Synthetic polypeptide"
DIVMTQSPATLSVTPGDRVSLSCRASQNFSDYLHWYQQKSHESPRLLIKYVSHSISGIPSRFSGSGSGSDFTLSINSVEPEDVGVYYCQNGHSFPPTFGGGTKLEIK

SEQ ID NO: 64 - protein, 116 aa, Artificial Sequence
  source: /note="Description of Artificial Sequence: Synthetic polypeptide"
QVQLQQSGAELVKPGASVKLSCKASGYTFTNYYIFWVKERPGQGLEWIGDINPSNGDTNFNEKFKIKATLTVDKSSSTTYMQLNSLTSEDSAVYFCTRGGYTMDYWGQGTSVTVSS

SEQ ID NO: 65 - protein, 112 aa, Artificial Sequence
  source: /note="Description of Artificial Sequence: Synthetic polypeptide"
DVVMTQTPLSLPVSLGDQASISCRSSQSLVHSNGNTYFHWYVQKPGQSPKLLIYKVSYRFSGVPDRFSGSGSGTDFTLKISRVEAEDLGVYFCSQSTHVPRTFGGGTKLEIK

SEQ ID NO: 66 - protein, 116 aa, Artificial Sequence
  source: /note="Description of Artificial Sequence: Synthetic polypeptide"
QVQLVQSGAEVKKPGASVKVSCKASGYTFTNYYIFWVRQAPGQGLEWIGDINPSNGDTNFNEKFKIKATLTVDKSTSTTYMELSSLRSEDTAVYYCTRGGYTMDYWGQGTLVTVSS

SEQ ID NO: 67 - protein, 116 aa, Artificial Sequence
  source: /note="Description of Artificial Sequence: Synthetic polypeptide"
QVQLVQSGAEVKKPGASVKVSCKASGYTFTNYYIFWVRQAPGQGLEWMGDINPSNGDTNFNEKFKIRVTMTRDTSTSTVYMELSSLRSEDTAVYYCTRGGYTMDYWGQGTLVTVSS

SEQ ID NO: 68 - protein, 112 aa, Artificial Sequence
  source: /note="Description of Artificial Sequence: Synthetic polypeptide"
DVVMTQTPLSLSVTPGQPASISCRSSQSLVHSNGNTYFHWYLQKPGQPPKLLIYKVSYRFSGVPDRFSGSGSGTDFTLKISRVEAEDVGVYFCSQSTHVPRTFGQGTKVEIK

SEQ ID NO: 69 - protein, 112 aa, Artificial Sequence
  source: /note="Description of Artificial Sequence: Synthetic polypeptide"
DIVMTQTPLSLSVTPGQPASISCRSSQSLVHSNGNTYFHWYLQKPGQPPQLLIYKVSYRFSGVPDRFSGSGSGTDFTLKISRVEAEDVGVYYCSQSTHVPRTFGQGTKVEIK

SEQ ID NO: 70 - protein, 118 aa, Artificial Sequence
  source: /note="Description of Artificial Sequence: Synthetic polypeptide"
EVQLQQSGAELVRSGASVKLSCTASGFNIKDYYLHWVKQRPEQGLEWIGWIDPDNGDTEFAPKFQGKATMTADTSSNTAYLQLSSLTSEDTAVYYCNAAYGSSSYPMDYWGQGTSVTV

SEQ ID NO: 71 - protein, 118 aa, Artificial Sequence
  source: /note="Description of Artificial Sequence: Synthetic polypeptide"
EVQLVQSGAEVKKPGATVKISCKVSGFNIKDYYLHWVQQAPGKGLEWMGWIDPDNGDTEYAEKFQGRVTITADTSTDTAYMELSSLRSEDTAVYYCNAAYGSSSYPMDYWGQGTTVTV

SEQ ID NO: 72 - protein, 118 aa, Artificial Sequence
  source: /note="Description of Artificial Sequence: Synthetic polypeptide"
QMQLVQSGAEVKKTGSSVKVSCKASGFNIKDYYLHWVRQAPGQALEWMGWIDPDNGDTEYAQKFQDRVTITRDRSMSTAYMELSSLRSEDTAMYYCNAAYGSSSYPMDYWGQGTTVTV

SEQ ID NO: 73 - protein, 118 aa, Artificial Sequence
  source: /note="Description of Artificial Sequence: Synthetic polypeptide"
EVQLVQSGAEVKKTGSSVKVSCKASGFNIKDYYLHWVRQAPGQALEWMGWIDPDNGDTEYAQKFQDRVTITRDRSMSTAYMELSSLRSEDTAMYYCNAAYGSSSYPMDYWGQGTTVTV

SEQ ID NO: 74 - protein, 118 aa, Artificial Sequence
  source: /note="Description of Artificial Sequence: Synthetic polypeptide"
QMQLVQSGAEVKKTGSSVKVSCKASGFNIKDYYLHWVRQAPGQALEWMGWIDPDNGDTEYAQKFQGRVTMTADTSSNTAYMELSSLRSEDTAMYYCNAAYGSSSYPMDYWGQGTTVTV

SEQ ID NO: 75 - protein, 118 aa, Artificial Sequence
  source: /note="Description of Artificial Sequence: Synthetic polypeptide"
QMQLVQSGAEVKKTGSSVKVSCKASGFNIKDYYLHWVRQAPGQALEWMGWIDPDNGDTEYAQKFQGRVTMTEDTSTDTAYMELSSLRSEDTAMYYCNAAYGSSSYPMDYWGQGTTVTV

SEQ ID NO: 76 - protein, 118 aa, Artificial Sequence
  source: /note="Description of Artificial Sequence: Synthetic polypeptide"
QMQLVQSGAEVKKTGSSVKVSCKASGFNIKDYYLHWVRQAPGQALEWMGWIDPDQGDTEYAQKFQDRVTITRDRSMSTAYMELSSLRSEDTAMYYCNAAYGSSSYPMDYWGQGTTVTV

SEQ ID NO: 77 - protein, 118 aa, Artificial Sequence
  source: /note="Description of Artificial Sequence: Synthetic polypeptide"
QMQLVQSGAEVKKTGSSVKVSCKASGFNIKDYYLHWVRQAPGQALEWMGWIDPDYGDTEYAQKFQDRVTITRDRSMSTAYMELSSLRSEDTAMYYCNAAYGSSSYPMDYWGQGTTVTV

SEQ ID NO: 78 - protein, 118 aa, Artificial Sequence
  source: /note="Description of Artificial Sequence: Synthetic polypeptide"
QMQLVQSGAEVKKTGSSVKVSCKASGFNIKDYYLHWVRQAPGQALEWMGWIDPDSGDTEYAQKFQDRVTITRDRSMSTAYMELSSLRSEDTAMYYCNAAYGSSSYPMDYWGQGTTVTV

SEQ ID NO: 79 - protein, 118 aa, Artificial Sequence
  source: /note="Description of Artificial Sequence: Synthetic polypeptide"
QMQLVQSGAEVKKTGSSVKVSCKASGFNIKDYYLHWVRQAPGQALEWMGWIDPDNADTEYAQKFQDRVTITRDRSMSTAYMELSSLRSEDTAMYYCNAAYGSSSYPMDYWGQGTTVTV

SEQ ID NO: 80 - protein, 118 aa, Artificial Sequence
  source: /note="Description of Artificial Sequence: Synthetic polypeptide"
QMQLVQSGAEVKKTGSSVKVSCKASGFNIKDYYLHWVRQAPGQALEWMGWIDPDNTDTEYAQKFQDRVTITRDRSMSTAYMELSSLRSEDTAMYYCNAAYGSSSYPMDYWGQGTTVTV

SEQ ID NO: 81 - protein, 118 aa, Artificial Sequence
  source: /note="Description of Artificial Sequence: Synthetic polypeptide"
QMQLVQSGAEVKKTGSSVKVSCKASGFNIKDYYLHWVRQAPGQALEWMGWIDPDNGDTEYAQKFQDRVTITRDRSMSTAYMELSSLRSEDTAMYYCNAAYGSSPYPMDYWGQGTTVTV

SEQ ID NO: 82 - protein, 118 aa, Artificial Sequence
  source: /note="Description of Artificial Sequence: Synthetic polypeptide"
QMQLVQSGAEVKKTGSSVKVSCKASGYTFTYYYLHWVRQAPGQALEWMGWIDPDNGDTEYAQKFQDRVTITRDRSMSTAYMELSSLRSEDTAMYYCNAAYGSSSYPMDYWGQGTTVTV

SEQ ID NO: 83 - protein, 118 aa, Artificial Sequence
  source: /note="Description of Artificial Sequence: Synthetic polypeptide"
QMQLVQSGAEVKKTGSSVKVSCKASGFTFTYYYLHWVRQAPGQALEWMGWIDPDNGDTEYAQKFQDRVTITRDRSMSTAYMELSSLRSEDTAMYYCNAAYGSSSYPMDYWGQGTTVTV

SEQ ID NO: 84 - protein, 118 aa, Artificial Sequence
  source: /note="Description of Artificial Sequence: Synthetic polypeptide"
QMQLVQSGAEVKKTGSSVKVSCKASGYNFTYYYLHWVRQAPGQALEWMGWIDPDNGDTEYAQKFQDRVTITRDRSMSTAYMELSSLRSEDTAMYYCNAAYGSSSYPMDYWGQGTTVTV

SEQ ID NO: 85 - protein, 118 aa, Artificial Sequence
  source: /note="Description of Artificial Sequence: Synthetic polypeptide"
QMQLVQSGAEVKKTGSSVKVSCKASGYTITYYYLHWVRQAPGQALEWMGWIDPDNGDTEYAQKFQDRVTITRDRSMSTAYMELSSLRSEDTAMYYCNAAYGSSSYPMDYWGQGTTVTV

SEQ ID NO: 86 - protein, 118 aa, Artificial Sequence
  source: /note="Description of Artificial Sequence: Synthetic polypeptide"
QMQLVQSGAEVKKTGSSVKVSCKASGYTFKYYYLHWVRQAPGQALEWMGWIDPDNGDTEYAQKFQDRVTITRDRSMSTAYMELSSLRSEDTAMYYCNAAYGSSSYPMDYWGQGTTVTV

SEQ ID NO: 87 - protein, 118 aa, Artificial Sequence
  source: /note="Description of Artificial Sequence: Synthetic polypeptide"
QMQLVQSGAEVKKTGSSVKVSCKASGYTFTDYYLHWVRQAPGQALEWMGWIDPDNGDTEYAQKFQDRVTITRDRSMSTAYMELSSLRSEDTAMYYCNAAYGSSSYPMDYWGQGTTVTV

SEQ ID NO: 88 - protein, 118 aa, Artificial Sequence
  source: /note="Description of Artificial Sequence: Synthetic polypeptide"
QMQLVQSGAEVKKTGSSVKVSCKASGFTFTDYYLHWVRQAPGQALEWMGWIDPDNGDTEYAQKFQDRVTITRDRSMSTAYMELSSLRSEDTAMYYCNAAYGSSSYPMDYWGQGTTVTV

SEQ ID NO: 89 - protein, 118 aa, Artificial Sequence
  source: /note="Description of Artificial Sequence: Synthetic polypeptide"
QMQLVQSGAEVKKTGSSVKVSCKASGFTITDYYLHWVRQAPGQALEWMGWIDPDNGDTEYAQKFQDRVTITRDRSMSTAYMELSSLRSEDTAMYYCNAAYGSSSYPMDYWGQGTTVTV

SEQ ID NO: 90 - protein, 118 aa, Artificial Sequence
  source: /note="Description of Artificial Sequence: Synthetic polypeptide"
QMQLVQSGAEVKKTGSSVKVSCKASGYTFKDYYLHWVRQAPGQALEWMGWIDPDNGDTEYAQKFQDRVTITRDRSMSTAYMELSSLRSEDTAMYYCNAAYGSSSYPMDYWGQGTTVTV

SEQ ID NO: 91 - protein, 118 aa, Artificial Sequence
  source: /note="Description of Artificial Sequence: Synthetic polypeptide"
QMQLVQSGAEVKKTGSSVKVSCKASGFTFKDYYLHWVRQAPGQALEWMGWIDPDNGDTEYAQKFQDRVTITRDRSMSTAYMELSSLRSEDTAMYYCNAAYGSSSYPMDYWGQGTTVTV

SEQ ID NO: 92 - protein, 118 aa, Artificial Sequence
  source: /note="Description of Artificial Sequence: Synthetic polypeptide"
QMQLVQSGAEVKKTGSSVKVSCKASGFNIKDYYLHWVRQAPGQALEWMGWIDPDNGDTEYAQKFQDRVTITRDRSMSTAYLQLSSLRSEDTAMYYCNAAYGSSSYPMDYWGQGTTVTV

SEQ ID NO: 93 - protein, 118 aa, Artificial Sequence
  source: /note="Description of Artificial Sequence: Synthetic polypeptide"
QMQLVQSGAEVKKTGSSVKVSCKASGFNIKDYYLHWVRQAPGQALEWMGWIDPDNGDTEYAQKFQDRVTITRDRSMSTAYMELSSLTSEDTAVYYCNAAYGSSSYPMDYWGQGTTVTV

SEQ ID NO: 94 - protein, 118 aa, Artificial Sequence
  source: /note="Description of Artificial Sequence: Synthetic polypeptide"
EVQLVQSGAEVKKPGATVKISCKVSGFNIKDYYLHWVRQAPGQALEWMGWIDPDNGDTEYAQKFQDRVTITRDRSMSTAYMELSSLRSEDTAMYYCNAAYGSSSYPMDYWGQGTTVTV

SEQ ID NO: 95 - protein, 118 aa, Artificial Sequence
  source: /note="Description of Artificial Sequence: Synthetic polypeptide"
EVQLVQSGAEVKKPGATVKISCKVSGFNIKDYYLHWVQQAPGKGLEWMGWIDPDNGDTEYAQKFQDRVTITRDRSMSTAYMELSSLRSEDTAMYYCNAAYGSSSYPMDYWGQGTTVTV

SEQ ID NO: 96 - protein, 107 aa, Artificial Sequence
  source: /note="Description of Artificial Sequence: Synthetic polypeptide"
DIKMTQSPSSLYASLGERVTITCKASQDIHRYLSWFQQKPGKSPKILIYRANRLVDGVPSRFSGSGSGQDYSLTISSLEYEDMGIYYCLQYDEFPYTFGGGTKLEMK

SEQ ID NO: 97 - protein, 107 aa, Artificial Sequence
  source: /note="Description of Artificial Sequence: Synthetic polypeptide"
DIKMTQSPSSLYASLGERVTITCKASQDIHRYLSWFQQKPGKSPKILIYRANRLVDGVPSRFSGSGSGQDYSLTISSLEYEDMGIYYCLQYDEFPYTFGGGTKLEIK

SEQ ID NO: 98 - protein, 107 aa, Artificial Sequence
  source: /note="Description of Artificial Sequence: Synthetic polypeptide"
DIQMTQSPSSLSASVGDRVTITCKASQDIHRYLSWYQQKPGKAPKLLIYRANRLVDGVPSRFSGSGSGTDFTFTISSLQPEDIATYYCLQYDEFPYTFGGGTKVEIK

SEQ ID NO: 99 - protein, 107 aa, Artificial Sequence
  source: /note="Description of Artificial Sequence: Synthetic polypeptide"
DIQMTQSPSSLSASVGDRVTITCKASQDIHRYLSWFQQKPGKAPKSLIYRANRLVDGVPSRFSGSGSGTDFTLTISSLQPEDFATYYCLQYDEFPYTFGGGTKVEIK

SEQ ID NO: 100 - protein, 107 aa, Artificial Sequence
  source: /note="Description of Artificial Sequence: Synthetic polypeptide"
NIQMTQSPSAMSASVGDRVTITCKASQDIHRYLSWFQQKPGKVPKHLIYRANRLVDGVPSRFSGSGSGTEFTLTISSLQPEDFATYYCLQYDEFPYTFGGGTKVEIK

SEQ ID NO: 101 - protein, 107 aa, Artificial Sequence
  source: /note="Description of Artificial Sequence: Synthetic polypeptide"
DIQMTQSPSSLSASVGDRVTITCKASQDIHRYLSWYQQKPGKAPKRLIYRANRLVDGVPSRFSGSGSGTEFTLTISSLQPEDFATYYCLQYDEFPYTFGGGTKVEIK

SEQ ID NO: 102 - protein, 107 aa, Artificial Sequence
  source: /note="Description of Artificial Sequence: Synthetic polypeptide"
DIQMTQSPSSLSASVGDRVTITCRASQDIHRYLAWYQQKPGKVPKLLIYRANRLQSGVPSRFSGSGSGTDFTLTISSLQPEDVATYYCLQYDEFPYTFGQGTKVEIK

SEQ ID NO: 103 - protein, 107 aa, Artificial Sequence
  source: /note="Description of Artificial Sequence: Synthetic polypeptide"
EIVLTQSPATLSLSPGERATLSCRASQDIHRYLAWYQQKPGQAPRLLIYRANRRATGIPARFSGSGSGTDFTLTISSLEPEDFAVYYCLQYDEFPYTGFQGTRLEIK

SEQ ID NO: 104 - protein, 107 aa, Artificial Sequence
  source: /note="Description of Artificial Sequence: Synthetic polypeptide"
DIQMTQSPSAMSASVGDRVTITCKASQDIHRYLSWFQQKPGKVPKHLIYRANRLVDGVPSRFSGSGSGTEFTLTISSLQPEDFATYYCLQYDEFPYTFGGGTKVEIK

SEQ ID NO: 105 - protein, 107 aa, Artificial Sequence
  source: /note="Description of Artificial Sequence: Synthetic polypeptide"
NIQMTQSPSAMSASVGDRVTITCRARQGIHRYLSWFQQKPGKVPKHLIYRANRLVDGVPSRFSGSGSGTEFTLTISSLQPEDFATYYCLQYDEFPYTFGGGTKVEIK

SEQ ID NO: 106 - protein, 107 aa, Artificial Sequence
  source: /note="Description of Artificial Sequence: Synthetic polypeptide"
NIQMTQSPSAMSASVGDRVTITCKASQDIHRYLSWFQQKPGKVPKILIYRANRLVDGVPSRFSGSGSGTEFTLTISSLQPEDFATYYCLQYDEFPYTFGGGTKVEIK

SEQ ID NO: 107 - protein, 107 aa, Artificial Sequence
  source: /note="Description of Artificial Sequence: Synthetic polypeptide"
NIQMTQSPSAMSASVGDRVTITCKASQDIHRYLSWFQQKPGKVPKHLIYRANRLVSGVPSRFSGSGSGTEFTLTISSLQPEDFATYYCLQYDEFPYTFGGGTKVEIK

SEQ ID NO: 108 - protein, 107 aa, Artificial Sequence
  source: /note="Description of Artificial Sequence: Synthetic polypeptide"
NIQMTQSPSAMSASVGDRVTITCRARQGIHRYLSWFQQKPGKVPKILIYRANRLVDGVPSRFSGSGSGTEFTLTISSLQPEDFATYYCLQYDEFPYTFGGGTKVEIK

SEQ ID NO: 109 - protein, 107 aa, Artificial Sequence
  source: /note="Description of Artificial Sequence: Synthetic polypeptide"
NIQMTQSPSAMSASVGDRVTITCRARQGIHRYLSWFQQKPGKVPKHLIYRANRLVSGVPSRFSGSGSGTEFTLTISSLQPEDFATYYCLQYDEFPYTFGGGTKVEIK

SEQ ID NO: 110 - protein, 107 aa, Artificial Sequence
  source: /note="Description of Artificial Sequence: Synthetic polypeptide"
NIQMTQSPSAMSASVGDRVTITCKASQDIHRYLSWFQQKPGKVPKLLIYRANRLVDGVPSRFSGSGSGTEFTLTISSLQPEDFATYYCLQYDEFPYTFGGGTKVEIK

SEQ ID NO: 111 - protein, 107 aa, Artificial Sequence
  source: /note="Description of Artificial Sequence: Synthetic polypeptide"
NIQMTQSPSAMSASVGDRVTITCKASQDIHRYLSWFQQKPGKVPKLLIYRANRLVSGVPSRFSGSGSGTEFTLTISSLQPEDFATYYCLQYDEFPYTFGGGTKVEIK

SEQ ID NO: 112 - protein, 107 aa, Artificial Sequence
  source: /note="Description of Artificial Sequence: Synthetic polypeptide"
NIQMTQSPSAMSASVGDRVTITCRARQGIHRYLSWFQQKPGKVPKLLIYRANRLVSGVPSRFSGSGSGTEFTLTISSLQPEDFATYYCLQYDEFPYTFGGGTKVEIK

SEQ ID NO: 113 - protein, 117 aa, Artificial Sequence
  source: /note="Description of Artificial Sequence: Synthetic polypeptide"
QVQLVQSGAEVKKPGASVKVSCKASGYTFTNYNMHWVRQAPGQGLEWIGTIYPGNDDTSYNQKFKDKATLTADKSTSTAYMELSSLRSEDTAVYYCARGGYRAMDYWGQGTLVTVSS

SEQ ID NO: 114 - protein, 117 aa, Artificial Sequence
  source: /note="Description of Artificial Sequence: Synthetic polypeptide"
QVQLVQSGAEVKKPGASVKVSCKASGYTFTNYNMHWVRQAPGQRLEWMGTIYPGNDDTSYNQKFKDRVTITADTSASTAYMELSSLRSEDTAVYYCARGGYRAMDYWGQGTLVTVSS

SEQ ID NO: 115 - protein, 117 aa, Artificial Sequence
  source: /note="Description of Artificial Sequence: Synthetic polypeptide"
QVQLVQSGAEVKKPGASVKVSCKASGYTFTNYNMHWVRQAPGQRLEWIGTIYPGNDDTSYNQKFKDRATLTADKSASTAYMELSSLRSEDTAVYYCARGGYRAMDYWGQGTLVTVSS

SEQ ID NO: 116 - protein, 112 aa, Artificial Sequence
  source: /note="Description of Artificial Sequence: Synthetic polypeptide"
DVVMTQSPLSLPVTPGEPASISCRSSQSIVYSNGNTYLGWYLQKPGQSPKLLIYKVSNRFSGVPDRFSGSGSGTDFTLKISRVEAEDVGVYHCFQGSHVPYTFGGGTKVEIK

SEQ ID NO: 117 - protein, 112 aa, Artificial Sequence
  source: /note="Description of Artificial Sequence: Synthetic polypeptide"
DIVMTQSPLSLPVTPGEPASISCRSSQSIVYSNGNTYLGWYLQKPGQSPQLLIYKVSNRFSGVPDRFSGSGSGTDFTLKISRVEAEDVGVYYCFQGSHVPYTFGQGTKLEIK

SEQ ID NO: 118 - protein, 112 aa, Artificial Sequence
  source: /note="Description of Artificial Sequence: Synthetic polypeptide"
DVVMTQSPLSLPVTPGEPASISCRSSQSIVYSNGNTYLGWYLQKPGQSPQLLIYKVSNRFSGVPDRFSGSGSGTDFTLKISRVEAEDVGVYHCFQGSHVPYTFGQGTKLEIK

SEQ ID NO: 119 - protein, 120 aa, Artificial Sequence
  source: /note="Description of Artificial Sequence: Synthetic polypeptide"
QVQLQQPGAELVRPGSSVKLSCKASGYTFTSYWVHWVKQRPIQGLEWIGNIDPSDSDTHYNQKFKDKASLTVDKSSSTAYMQLSSLTFEDSAVYYCVRGGTGTMAWFAYWGQGTLVTVSA

SEQ ID NO: 120 - protein, 120 aa, Artificial Sequence
  source: /note="Description of Artificial Sequence: Synthetic polypeptide"
EVQLVQSGAEVKKPGESLRISCKASGYTFTSYWVHWVRQMPGKGLEWIGNIDPSDSDTHYNQKFKDHVTLSVDKSISTAYLQLSSLKASDTAMYYCVRGGTGTMAWFAYWGQGTLVTVSS

SEQ ID NO: 121 - protein, 120 aa, Artificial Sequence
  source: /note="Description of Artificial Sequence: Synthetic polypeptide"
EVQLVQSGAEVKKPGESLRISCKASGYSFTSYWVHWVRQMPGKGLEWMGNIDPSDSDTHYNQKFKDHVTLSVDKSISTAYLQLSSLKASDTAMYYCVRGGTGTMAWFAYWGQGTLVTVSS

SEQ ID NO: 122 - protein, 120 aa, Artificial Sequence
  source: /note="Description of Artificial Sequence: Synthetic polypeptide"
EVQLVQSGAEVKKPGESLRISCKASGYSFTSYWVHWVRQMPGKGLEWMGNIDPSDSDTHYSPSFQGHVTLSVDKSISTAYLQLSSLKASDTAMYYCVRGGTGTMAWFAYWGQGTLVTVSS

SEQ ID NO: 123 - protein, 120 aa, Artificial Sequence
  source: /note="Description of Artificial Sequence: Synthetic polypeptide"
EVQLVQSGAEVKKPGESLRISCKASGYSFTSYWVHWVRQMPGKGLEWMGNIDPSDSDTHYSPSFQGHVTLSVDKSISTAYLQLSSLKASDTAMYYCVRGGTGTLAWFAYWGQGTLVTVSS

SEQ ID NO: 124 - protein, 120 aa, Artificial Sequence
  source: /note="Description of Artificial Sequence: Synthetic polypeptide"
EVQLVQSGAEVKKPGESLRISCKASGYSFTSYWVHWVRQMPGKGLEWMGNIDPSDSDTHYSPSFQGHVTLSVDKSISTAYLQLSSLKASDTAMYYCVRGGTGTMAYFAYWGQGTLVTVSS

SEQ ID NO: 125 - protein, 120 aa, Artificial Sequence
  source: /note="Description of Artificial Sequence: Synthetic polypeptide"
EVQLVQSGAEVKKPGESLRISCKASGYSFTSYWVHWVRQMPGKGLEWMGNIDPSDSDTHYSPSFQGHVTLSVDKSISTAYLQLSSLKASDTAMYYCVRGGTGTLAYFAYWGQGTLVTVSS

SEQ ID NO: 126 - protein, 112 aa, Artificial Sequence
  source: /note="Description of Artificial Sequence: Synthetic polypeptide"
DVVMTQTPLSLPVSLGDQASISCRSSQSLVHSYGNTYLYWYLQKPGQSPKLLIYRVSNRFSGVPDRFSGSGSGTDFTLKISRVEAEDLGVYFCFQGTHVPYTFGSGTKLEIK

SEQ ID NO: 127 - protein, 112 aa, Artificial Sequence
  source: /note="Description of Artificial Sequence: Synthetic polypeptide"
DVVMTQSPLSLPVTLGQPASISCRSSQSLVHSYGNTYLYWYQQRPGQSPRLLIYRVSNRFSGVPDRFSGSGSGTDFTLKISRVEAEDVGVYFCFQGTHVPYTFGGGTKVEIK

SEQ ID NO: 128 - protein, 112 aa, Artificial Sequence
  source: /note="Description of Artificial Sequence: Synthetic polypeptide"
DVVMTQSPLSLPVTLGQPASISCRSSQSLVHSYGNTYLYWFQQRPGQSPRLLIYRVSNRFSGVPDRFSGSGSGTDFTLKISRVEAEDVGVYYCFQGTHVPYTFGGGTKVEIK

SEQ ID NO: 129 - protein, 393 aa, Homo sapiens [sequence omitted]

SEQ ID NO: 130 - DNA, 2512 bp, Homo sapiens
ctcaaaagtctagagccaccgtccagggagcaggtagctgctgggctccggggacactttgcgttcgggctgggagcgtgctttccacgacggtgacacgcttccctggattggcagccagactgccttccgggtcactgccatggaggagccgcagtcagatcctagcgtcgagccccctctgagtcaggaaacattttcagacctatggaaactacttcctgaaaacaacgttctgtcccccttgccgtcccaagcaatggatgatttgatgctgtccccggacgatattgaacaatggttcactgaagacccaggtccagatgaagctcccagaatgccagaggctgctccccccgtggcccctgcaccagcagctcctacaccggcggcccctgcaccagccccctcctggcccctgtcatcttctgtcccttcccagaaaacctaccagggcagctacggtttccgtctgggcttcttgcattctgggacagccaagtctgtgacttgcacgtactcccctgccctcaacaagatgttttgccaactggccaagacctgccctgtgcagctgtgggttgattccacacccccgcccggcacccgcgtccgcgccatggccatctacaagcagtcacagcacatgacggaggttgtgaggcgctgcccccaccatgagcgctgctcagatagcgatggtctggcccctcctcagcatcttatccgagtggaaggaaatttgcgtgtggagtatttggatgacagaaacacttttcgacatagtgtggtggtgccctatgagccgcctgaggttggctctgactgtaccaccatccactacaactacatgtgtaacagttcctgcatgggcggcatgaaccggaggcccatcctcaccatcatcacactggaagactccagtggtaatctactgggacggaacagctttgaggtgcgtgtttgtgcctgtcctgggagagaccggcgcacagaggaagagaatctccgcaagaaaggggagcctcaccacgagctgcccccagggagcactaagcgagcactgcccaacaacaccagctcctctccccagccaaagaagaaaccactggatggagaatatttcacccttcagatccgtgggcgtgagcgcttcgagatgttccgagagctgaatgaggccttggaactcaaggatgcccaggctgggaaggagccaggggggagcagggctcactccagccacctgaagtccaaaaagggtcagtctacctcccgccataaaaaactcatgttcaagacagaagggcctgactcagactgacattctccacttcttgttccccactgacagcctcccacccccatctctccctcccctgccattttgggttttgggtctttgaacccttgcttgcaataggtgtgcgtcagaagcacccaggacttccatttgctttgtcccggggctccactgaacaagttggcctgcactggtgttttgttgtggggaggaggatggggagtaggacataccagcttagattttaaggtttttactgtgagggatgtttgggagatgtaagaaatgttcttgcagttaagggttagtttacaatcagccacattctaggtaggggcccacttcaccgtactaaccagggaagctgtccctcactgttgaattttctctaacttcaaggcccatatctgtgaaatgctggcatttgcacctacctcacagagtgcattgtgagggttaatgaaataatgtacatctggccttgaaaccaccttttattacatggggtctagaacttgacccccttgagggtgcttgttccctctccctgttggtcggtgggttggtagtttctacagttgggcagctggttaggtagagggagttgtcaagtctctgctggcccagccaaaccctgtctgacaacctcttggtgaaccttagtacctaaaaggaaatctcaccccatcccacaccctggaggatttcatctcttgtatatgatgatctggatccaccaagacttgttttatgctcagggtcaatttcttttttcttttttttttttttttttctttttctttgagactgggtctcgctttgttgcccaggctggagtggagtggcgtgatcttggcttactgcagcctttgcctccccggctcgagcagtcctgcctcagcctccggagtagctgggaccacaggttcatgccaccatggccagccaacttttgcatgttttgtagagatggggtctcacagtgttgcccaggctggtctcaaactcctgggctcaggcgatccacctgtctcagcctcccagagtgctgggattacaattgtgagccaccacgtccagctggaagggtcaacatcttttacattctgcaagcacatctgcattttcaccccacccttcccctccttctccctttttatatcccatttttatatcgatctcttattttacaataaaactttgctgcca

SEQ ID NO: 131 - protein, 117 aa, Artificial Sequence; identical to SEQ ID NO: 114
  source: /note="Description of Artificial Sequence: Synthetic polypeptide"

SEQ ID NO: 132 - protein, 112 aa, Artificial Sequence; identical to SEQ ID NO: 117
  source: /note="Description of Artificial Sequence: Synthetic polypeptide"

SEQ ID NO: 133 - protein, 16 aa, Artificial Sequence
  source: /note="Description of Artificial Sequence: Synthetic peptide"
RSSQSIVYSNGNTYLG

SEQ ID NO: 134 - protein, 8 aa, Artificial Sequence
  source: /note="Description of Artificial Sequence: Synthetic peptide"
GYTFTNYN

SEQ ID NO: 135 - protein, 8 aa, Artificial Sequence
  source: /note="Description of Artificial Sequence: Synthetic peptide"
IYPGNDDT

SEQ ID NO: 136 - protein, 10 aa, Artificial Sequence
  source: /note="Description of Artificial Sequence: Synthetic peptide"
ARGGYRAMDY

SEQ ID NO: 137 - protein, 11 aa, Artificial Sequence
  source: /note="Description of Artificial Sequence: Synthetic peptide"
QSIVYSNGNTY

SEQ ID NO: 138 - protein, 3 aa, Artificial Sequence
  source: /note="Description of Artificial Sequence: Synthetic peptide"
KVS

SEQ ID NO: 139 - protein, 9 aa, Artificial Sequence
  source: /note="Description of Artificial Sequence: Synthetic peptide"
FQGSHVPYT

SEQ ID NO: 140 - protein, 7 aa, Artificial Sequence
  source: /note="Description of Artificial Sequence: Synthetic peptide"
GYTFTNY

SEQ ID NO: 141 - protein, 4 aa, Artificial Sequence
  source: /note="Description of Artificial Sequence: Synthetic peptide"
PGND

SEQ ID NO: 142 - protein, 6 aa, Artificial Sequence
  source: /note="Description of Artificial Sequence: Synthetic peptide"
GYRAMD

SEQ ID NO: 143 - protein, 12 aa, Artificial Sequence
  source: /note="Description of Artificial Sequence: Synthetic peptide"
SQSIVYSNGNTY

SEQ ID NO: 144 - protein, 3 aa, Artificial Sequence
  source: /note="Description of Artificial Sequence: Synthetic peptide"
KVS

SEQ ID NO: 145 - protein, 6 aa, Artificial Sequence
  source: /note="Description of Artificial Sequence: Synthetic peptide"
GSHVPY

SEQ ID NO: 146 - protein, 10 aa, Artificial Sequence
  source: /note="Description of Artificial Sequence: Synthetic peptide"
ASGYTFTNYN

SEQ ID NO: 147 - protein, 17 aa, Artificial Sequence
  source: /note="Description of Artificial Sequence: Synthetic peptide"
IYPGNDDTSYNQKFKDR

SEQ ID NO: 148 - protein, 7 aa, Artificial Sequence
  source: /note="Description of Artificial Sequence: Synthetic peptide"
GGYRAMD

SEQ ID NO: 149 - protein, 13 aa, Artificial Sequence
  source: /note="Description of Artificial Sequence: Synthetic peptide"
SSQSIVYSNGNTY

SEQ ID NO: 150 - protein, 12 aa, Artificial Sequence
  source: /note="Description of Artificial Sequence: Synthetic peptide"
KVSNRFSGVPDR

SEQ ID NO: 151 - protein, 6 aa, Artificial Sequence
  source: /note="Description of Artificial Sequence: Synthetic peptide"
GSHVPY

SEQ ID NO: 152 - protein, 15 aa, Artificial Sequence
  source: /note="Description of Artificial Sequence: Synthetic peptide"
RRCPLYISYDPVCRR

SEQ ID NO: 153 - protein, 19 aa, Artificial Sequence
  source: /note="Description of Artificial Sequence: Synthetic peptide"
RRRRCPLYISYDPVCRRRR